European Patent Specification EP 4 106 871 B1, published March 13, 2024. Title: Biphenyl compounds as SOCE modulators, compositions and uses thereof. Applicant: Unversità degli Studi del Piemonte Orientale "Amedeo Avogadro". The sequence listing filed with the application follows.

SEQUENCE LISTING (2 sequences)

SEQ ID NO: 1 - DNA, 18 bp, artificial
  forward F118.20 primer
tgccagtttccctatcag

SEQ ID NO: 2 - DNA, 20 bp, artificial
  reverse F118.21 primer
cctaaggatgggatgtaacc